European Patent Specification EP 3 565 636 B1, published January 3, 2024. Title: USE OF GUT MICROBIOTA IN THE DIAGNOSIS AND THERAPEUTICS OF PARKINSON'S DISEASE. Applicant: California Institute of Technology Mazmanian, Sarkis K. Sampson, Timothy R. The sequence listing filed with the application follows.

SEQUENCE LISTING (8 sequences)

SEQ ID NO: 1 - protein, 151 aa, Escherichia coli
  VARIANT (1)...(151): CsgA from strain K-12
  ref <308>: Genbank No. CQR80619
  ref <309>: 2015-04-02
MKLLKVAAIAAIVFSGSALAGVVPQYGGGGNHGGGGNNSGPNSELNIYQYGGGNSALALQTDARNSDLTITQHGGGNGADVGQGSDDSSIDLTQRGFGNSATLDQWNGKNSEMTVKQFGGGNGAAVDQTASNSSVNVTQVGFGNNATAHQY

SEQ ID NO: 2 - protein, 152 aa, Escherichia coli
  VARIANT (1)...(152): CsgA from strain H8824
  ref <308>: Genbank No. EU554560
  ref <309>: 2008-12-02
MKLLKVAAIAAIVFSGSALAGVVPQYGGGGGNHGGGGNNSGPNSELNIYQYGGGNSALALQADARNSDLTITQHGGGNGADVGQGSDDSSIDLTQRGFGNSATLDQWNGKDSHMTVKQFGGGNGAAVDQTASNSTVNVTQVGFGNNATAHQY

SEQ ID NO: 3 - protein, 152 aa, Escherichia coli; identical to SEQ ID NO: 2
  VARIANT (1)...(152): CsgA from strain E06/486
  ref <308>: Genbank No. EU554559
  ref <309>: 2008-12-02

SEQ ID NO: 4 - protein, 152 aa, Escherichia coli; identical to SEQ ID NO: 2
  VARIANT (1)...(152): CsgA from strain 080/01
  ref <308>: Genbank No. EU554558
  ref <309>: 2008-12-02

SEQ ID NO: 5 - protein, 152 aa, Escherichia coli; identical to SEQ ID NO: 2
  VARIANT (1)...(152): CsgA from strain 340/97
  ref <308>: Genbank No. EU554557
  ref <309>: 2008-12-02

SEQ ID NO: 6 - protein, 151 aa, Enterobacter cloacae
  VARIANT (1)...(151): CsgA
  ref <308>: Genbank No. EF490314
  ref <309>: 2007-05-07
MKLFKVAVIAAIVVSGSAFAGAVPQFGGGHGGGWGGGNNGPDSTLSIYQYGGGNSALALQTDARDSELTITQHGGGNGADVGQGSDDSSIDLLQKGFGNSATIDQWNSKDSVINVKQFGGGNGAAVDQTASGSTVTVHQVGFGNNATAHQY

SEQ ID NO: 7 - protein, 173 aa, Stigmatella aurantiaca
  VARIANT (1)...(173): CsgA
  ref <308>: Genbank No. M95300.1
  ref <309>: 1993-04-26
MRAFASAVSDGPLDVLINNAGVSGKWCSFMEMDYEDMTKVMETNSVGPMRLSAALMPAVLKGPTRKIIHLTTRMASLTENTRGGVYGFEGGAYAYRMSKAALNVCMRTMAVDFRDQGLITAAINPGWVRTEMGGKLAPMRPEDAVRGMLRVIDDITKEQSGMFLDFQGREVPW

SEQ ID NO: 8 - protein, 151 aa, Escherichia coli; identical to SEQ ID NO: 1
  VARIANT (1)...(151): CsgA from strain K-12 substrain MC4100
  ref <308>: Genbank No. CDJ71478
  ref <309>: 2015-02-27